European Patent Specification EP 3 741 218 B1, published May 14, 2025. Title: LACTOBACILLUS SALIVARUS STRAIN AND ITS USE IN THE PREVENTION AND TREATMENT OF POST-WEANING DIARRHEA. Applicant: PROBISEARCH, S.L.U. The sequence listing filed with the application follows.

SEQUENCE LISTING (3 sequences)

SEQ ID NO: 1 - DNA, 20 bp, Artificial Sequence
  Primer plb16
agagtttgatcctggctcag

SEQ ID NO: 2 - DNA, 20 bp, Artificial Sequence
  Primer mlb16
ggctgctggcacgtagttag

SEQ ID NO: 3 - DNA, 505 bp, Lactobacillus salivarius
ttaaacgtcatcgatgacagttactctcactcgtgttcttctctaacaacagagttttacgatccgaagaccttcttcactcacgcggcgttgctccatcagacttgcgtccattgtggaagattccctactgctgcctcccgtaggagtttgggccgtgtctcagtcccaatgtggccgatcaacctctcagttcggctacgtatcatcaccttggtaggccgttaccccaccaactagttaatacgccgcgggtccatctaaaagcgatagcagaaccatctttcatctaaggatcatgcgatccttagagatatacggtattagcacctgtttccaagtgttatccccttcttttaggcaggttacccacgtgttactcacccgtccgccactcaacttcttacggtgaatgcaagcattcggtgtaagaaagtttcgttcgacttgcatgtattaggcacgccgccagcgttcgtcctgagccaggatccaaactcaaaaa